European Patent Specification EP 3 498 263 B1, published November 29, 2023. Title: Stable Liquid Pharmaceutical Formulation of Anti-Influenza Virus Antibody. Applicant: CELLTRION INC. The sequence listing filed with the application follows.

SEQUENCE LISTING (140 sequences)

SEQ ID NO: 1 - protein, 11 aa, Artificial Sequence
  Antibody 1 light chain CDR1
RASENIWNNLA

SEQ ID NO: 2 - protein, 7 aa, Artificial Sequence
  Antibody 1 light chain CDR2
GASTGAT

SEQ ID NO: 3 - protein, 9 aa, Artificial Sequence
  Antibody 1 light chain CDR3
QQYNSWPRT

SEQ ID NO: 4 - protein, 5 aa, Artificial Sequence
  Antibody 1 heavy chain CDR1
SHAIS

SEQ ID NO: 5 - protein, 17 aa, Artificial Sequence
  Antibody 1 heavy chain CDR2
GISPMFGTTHYAQKFQG

SEQ ID NO: 6 - protein, 14 aa, Artificial Sequence
  Antibody 1 heavy chain CDR3
DGAGSYYPLNWFDP

SEQ ID NO: 7 - protein, 12 aa, Artificial Sequence
  Antibody 2 light chain CDR1
RASHRVGSTYIA

SEQ ID NO: 8 - protein, 7 aa, Artificial Sequence
  Antibody 2 light chain CDR2
GASNRAT

SEQ ID NO: 9 - protein, 9 aa, Artificial Sequence
  Antibody 2 light chain CDR3
QQFSVSPWT

SEQ ID NO: 10 - protein, 5 aa, Artificial Sequence
  Antibody 2 heavy chain CDR1
TYGVS

SEQ ID NO: 11 - protein, 17 aa, Artificial Sequence
  Antibody 2 heavy chain CDR2
WISAYTGITDYAQKFQG

SEQ ID NO: 12 - protein, 17 aa, Artificial Sequence
  Antibody 2 heavy chain CDR3
DKVQGRVEVGSGGRHDY

SEQ ID NO: 13 - protein, 12 aa, Artificial Sequence
  Antibody 3 light chain CDR1
RASQSLSSSSLV

SEQ ID NO: 14 - protein, 7 aa, Artificial Sequence
  Antibody 3 light chain CDR2
GASSRAT

SEQ ID NO: 15 - protein, 9 aa, Artificial Sequence
  Antibody 3 light chain CDR3
QQYGNSPYT

SEQ ID NO: 16 - protein, 6 aa, Artificial Sequence
  Antibody 3 heavy chain CDR1
NNYAIS

SEQ ID NO: 17 - protein, 18 aa, Artificial Sequence
  Antibody 3 heavy chain CDR2
GGISPIFGTLNYAERFQG

SEQ ID NO: 18 - protein, 11 aa, Artificial Sequence
  Antibody 3 heavy chain CDR3
GCGYNCYYFDG

SEQ ID NO: 19 - protein, 12 aa, Artificial Sequence
  Antibody 4 light chain CDR1
RASQSVSISYLA

SEQ ID NO: 20 - protein, 7 aa, Artificial Sequence
  Antibody 4 light chain CDR2
GASRRAT

SEQ ID NO: 21 - protein, 9 aa, Artificial Sequence
  Antibody 4 light chain CDR3
QQYGSSPYT

SEQ ID NO: 22 - protein, 5 aa, Artificial Sequence
  Antibody 4 heavy chain CDR1
RFGIH

SEQ ID NO: 23 - protein, 17 aa, Artificial Sequence
  Antibody 4 heavy chain CDR2
VIWYDGSNKFYADSVKG

SEQ ID NO: 24 - protein, 18 aa, Artificial Sequence
  Antibody 4 heavy chain CDR3
DSRGYCSSIICFEGGLDN

SEQ ID NO: 25 - protein, 12 aa, Artificial Sequence
  Antibody 5 light chain CDR1
RASRRVGSTYLA

SEQ ID NO: 26 - protein, 7 aa, Artificial Sequence
  Antibody 5 light chain CDR2
GASSRAA

SEQ ID NO: 27 - protein, 9 aa, Artificial Sequence
  Antibody 5 light chain CDR3
QQYAASPWT

SEQ ID NO: 28 - protein, 5 aa, Artificial Sequence
  Antibody 5 heavy chain CDR1
TYGIS

SEQ ID NO: 29 - protein, 17 aa, Artificial Sequence
  Antibody 5 heavy chain CDR2
WISAYTGNTDYAQKVQG

SEQ ID NO: 30 - protein, 17 aa, Artificial Sequence
  Antibody 5 heavy chain CDR3
DKVQGRVEAGSGGRHDY

SEQ ID NO: 31 - protein, 12 aa, Artificial Sequence
  Antibody 6 light chain CDR1
RASHSVGSTYIA

SEQ ID NO: 32 - protein, 7 aa, Artificial Sequence
  Antibody 6 light chain CDR2
GASNRAT

SEQ ID NO: 33 - protein, 9 aa, Artificial Sequence
  Antibody 6 light chain CDR3
QQFSVSPWT

SEQ ID NO: 34 - protein, 5 aa, Artificial Sequence
  Antibody 6 heavy chain CDR1
TYGVS

SEQ ID NO: 35 - protein, 17 aa, Artificial Sequence
  Antibody 6 heavy chain CDR2
WISGYTGITDYAQKSQG

SEQ ID NO: 36 - protein, 17 aa, Artificial Sequence
  Antibody 6 heavy chain CDR3
DKVQGRVEAGSGGRHDY

SEQ ID NO: 37 - protein, 12 aa, Artificial Sequence
  Antibody 7 light chain CDR1
RASHSIGSTYIA

SEQ ID NO: 38 - protein, 7 aa, Artificial Sequence
  Antibody 7 light chain CDR2
GASNRAS

SEQ ID NO: 39 - protein, 9 aa, Artificial Sequence
  Antibody 7 light chain CDR3
QQFSVSPWT

SEQ ID NO: 40 - protein, 5 aa, Artificial Sequence
  Antibody 7 heavy chain CDR1
TYGVS

SEQ ID NO: 41 - protein, 17 aa, Artificial Sequence
  Antibody 7 heavy chain CDR2
WISGYTGITDYAQKFQG

SEQ ID NO: 42 - protein, 17 aa, Artificial Sequence
  Antibody 7 heavy chain CDR3
DKVQGRVEVGSGGRHDY

SEQ ID NO: 43 - protein, 127 aa, Artificial Sequence
  Antibody 1 light chain variable region
MEAPAQLLFLLLLWLPDTTGEIVLTQSPATLSLSPGERATLSCRASENIWNNLAWYQQKPGQAPRLLISGASTGATGVPSRFRGSGSRTEFTLTISSLQSEDFAIYFCQQYNSWPRTFGPGTKVEIK

SEQ ID NO: 44 - protein, 142 aa, Artificial Sequence
  Antibody 1 heavy chain variable region
MDWTWRFLFVVAAATGVQCQVQLVQSGAEVKMPGSSVKVSCKTSGVFFSSHAISWVRQAPGQGLEWMGGISPMFGTTHYAQKFQGRVTITADQSTTTAYMELTSLTSEDTAVYYCARDGAGSYYPLNWFDPWGQGTLVTVSS

SEQ ID NO: 45 - protein, 108 aa, Artificial Sequence [sequence omitted]

SEQ ID NO: 46 - protein, 126 aa, Artificial Sequence [sequence omitted]

SEQ ID NO: 47 - protein, 128 aa, Artificial Sequence
  Antibody 3 light chain variable region
METPAQLLFLLLLWLPDTTGEIVLTQSPGTLSLSPGERATLSCRASQSLSSSSLVWYQQKPGQAPRLLIYGASSRATGIPDRFSGSGSGTDFTLTISRLEPEDFAVYYCQQYGNSPYTFGQGTQVEIK

SEQ ID NO: 48 - protein, 139 aa, Artificial Sequence
  Antibody 3 heavy chain variable region
MDWTWRFLFVVAAATGVQSQVQLVQSGAEVKKPGSSVKVSCKASGGTLNNYAISWVRQAPGQGLEWMGGISPIFGTLNYAERFQGRVTITADVFTNTVYMELSSLRSEDTAVYFCARGCGYNCYYFDGWGQGTLVTVSS

SEQ ID NO: 49 - protein, 128 aa, Artificial Sequence
  Antibody 4 light chain variable region
METPAQLLFLLLLWLPDTTGETVLTQSPGTLSLSPGERATLSCRASQSVSISYLAWYQRKPGQAPRLLIYGASRRATGIPDRFSGSGSGTDFTLTISRLEPEDFAVYYCQQYGSSPYTFGQGTKLEIK

SEQ ID NO: 50 - protein, 146 aa, Artificial Sequence
  Antibody 4 heavy chain variable region
MEFGLSWVFLVALLRGVQCQVQLVESGGGVVQPGRSLRLSCAASGFTFSRFGIHWVRQAPGKGLEWMAVIWYDGSNKFYADSVKGRFTISRDNSKNTVYLQMNSLRAEDTAVYYCAKDSRGYCSSIICFEGGLDNWGQGTLVTVSS

SEQ ID NO: 51 - protein, 108 aa, Artificial Sequence
  Antibody 5 light chain variable region
EIVLTQSPGTLSVSPGERATLSCRASRRVGSTYLAWYQQKPGQAPRRLIYGASSRAAGIPDRFSGTGSGTDFTLTISRVDPEDFAVYYCQQYAASPWTFGQGTTVEIK

SEQ ID NO: 52 - protein, 126 aa, Artificial Sequence
  Antibody 5 heavy chain variable region
QVQLVQSGGELKKPGASVRVSCKASGYTFTTYGISWVRQAPGQGLEWVGWISAYTGNTDYAQKVQGRVTMTTDTSTSTAYMELRSLTSDDTAVYYCARDKVQGRVEAGSGGRHDYWGQGTLVTVSS

SEQ ID NO: 53 - protein, 108 aa, Artificial Sequence
  Antibody 6 light chain variable region
EVVLTQSPGTLTLPPGDRATLSCRASHSVGSTYIAWFQQKSGQAPRRLIYGASNRATDIPDRFSGSGSGTDFTLTIRRLEPEDSAVYYCQQFSVSPWTFGQGTRVEIK

SEQ ID NO: 54 - protein, 126 aa, Artificial Sequence
  Antibody 6 heavy chain variable region
QVQLVQSGVEVKKPGASVKVSCKTSGYPFSTYGVSWVRQAPGQGLEWVGWISGYTGITDYAQKSQGRVTLTTDASTATAFLELRSLRPDDTATYFCARDKVQGRVEAGSGGRHDYWGQGTLVIVSS

SEQ ID NO: 55 - protein, 108 aa, Artificial Sequence
  Antibody 7 light chain variable region
EVVLTQSPGTLALPPGERATLSCRASHSIGSTYIAWYQQKSGQAPRRLIYGASNRASDIPDRFSGSGSGTDFTLTIRRLEPEDSAVYYCQQFSVSPWTFGQGTRVEIK

SEQ ID NO: 56 - protein, 126 aa, Artificial Sequence
  Antibody 7 heavy chain variable region
QVQLVQSGAEVKKPGASVKVSCKTSGYSFSTYGVSWVRQAPGQGLEWVGWISGYTGITDYAQKFQGRVTLTTDATTATAFLELRSLRPDDTATYFCARDKVQGRVEVGSGGRHDYWGQGTLVIVSS

SEQ ID NO: 57 - protein, 234 aa, Artificial Sequence
  Antibody 1 light chain
MEAPAQLLFLLLLWLPDTTGEIVLTQSPATLSLSPGERATLSCRASENIWNNLAWYQQKPGQAPRLLISGASTGATGVPSRFRGSGSRTEFTLTISSLQSEDFAIYFCQQYNSWPRTFGPGTKVEIKRTVAAPSVFIFPPSDEQLKSGTASVVCLLNNFYPREAKVQWKVDNALQSGNSQESVTEQDSKDSTYSLSSTLTLSKADYEKHKVYACEVTHQGLSSPVTKSFNRGEC

SEQ ID NO: 58 - protein, 472 aa, Artificial Sequence
  Antibody 1 heavy chain
MDWTWRFLFVVAAATGVQCQVQLVQSGAEVKMPGSSVKVSCKTSGVFFSSHAISWVRQAPGQGLEWMGGISPMFGTTHYAQKFQGRVTITADQSTTTAYMELTSLTSEDTAVYYCARDGAGSYYPLNWFDPWGQGTLVTVSSASTKGPSVFPLAPSSKSTSGGTAALGCLVKDYFPEPVTVSWNSGALTSGVHTFPAVLQSSGLYSLSSVVTVPSSSLGTQTYICNVNHKPSNTKVDKRVEPKSCDKTHTCPPCPAPELLGGPSVFLFPPKPKDTLMISRTREVTCVVVDVSHEDPEVKFNWYVDGVEVHNAKTKPREEQYNSTYRVVSVLTVLHQDWLNGKEYKCKVSNKALPAPIEKTISKAKGQPREPQVYTLPPSRDELTKNQVSLTCLVKGFYPSDIAVEWESNGQPENNYKTTPPVLDSDGSFFLYSKLTVDKSRWQQGNVFSCSVMHEGLHNHYTQKSLSLFPGK

SEQ ID NO: 59 - protein, 215 aa, Artificial Sequence
  Antibody 2 light chain
EVVLTQSPGTLALPPGERATLSCRASHRVGSTYIAWYQQKSGQAPRRLIYGASNRATDIPDRFSGSGSGTDFTLTIRRLEPEDSAVYYCQQFSVSPWTFGQGTRVEIKRTVAAPSVFIFPPSDEQLKSGTASVVCLLNNFYPREAKVQWKVDNALQSGNSQESVTEQDSKDSTYSLSSTLTLSKADYEKHKVYACEVTHQGLSSPVTKSFNRGEC

SEQ ID NO: 60 - protein, 456 aa, Artificial Sequence
  Antibody 2 heavy chain
QVQLVQSGAEVKKPGASVKVSCKTSGYSFSTYGVSWVRQAPGQGPEWVGWISAYTGITDYAQKFQGRVTLTTDATTATAFLDLRSLRPDDTATYFCARDKVQGRVEVGSGGRHDYWGQGTLVIVSSASTKGPSVFPLAPSSKSTSGGTAALGCLVKDYFPEPVTVSWNSGALTSGVHTFPAVLQSSGLYSLSSVVTVPSSSLGTQTYICNVNHKPSNTKVDKKVEPKSCDKTHTCPPCPAPELLGGPSVFLFPPKPKDTLMISRTPEVTCVVVDVSHEDPEVKFNWYVDGVEVHNAKTKPREEQYNSTYRVVSVLTVLHQDWLNGKEYKCKVSNKALPAPIEKTISKAKGQPREPQVYTLPPSRDELTKNQVSLTCLVKGFYPSDIAVEWESNGQPENNYKTTPPVLDSDGSFFLYSKLTVDKSRWQQGNVFSCSVMHEGLHNHYTQKSLSLSPGK

SEQ ID NO: 61 - protein, 235 aa, Artificial Sequence
  Antibody 3 light chain
METPAQLLFLLLLWLPDTTGEIVLTQSPGTLSLSPGERATLSCRASQSLSSSSLVWYQQKPGQAPRLLIYGASSRATGIPDRFSGSGSGTDFTLTISRLEPEDFAVYYCQQYGNSPYTFGQGTQVEIKRTVAAPSVFIFPPSDEQLKSGTASVVCLLNNFYPREAKVQWKVDNALQSGNSQESVTEQDSKDSTYSLSSTLTLSKADYEKHKVYACEVTHQGLSSPVTKSFNRGEC

SEQ ID NO: 62 - protein, 469 aa, Artificial Sequence
  Antibody 3 heavy chain
MDWTWRFLFVVAAATGVQSQVQLVQSGAEVKKPGSSVKVSCKASGGTLNNYAISWVRQAPGQGLEWMGGISPIFGTLNYAERFQGRVTITADVFTNTVYMELSSLRSEDTAVYFCARGCGYNCYYFDGWGQGTLVTVSSASTKGPSVFPLAPSSKSTSGGTAALGCLVKDYFPEPVTVSWNSGALTSGVHTFPAVLQSSGLYSLSSVVTVPSSSLGTQTYICNVNHKPSNTKVDKKVEPKSCDKTHTCPPCPAPELLGGPSVFLFPPKPKDTLMISRTPEVTCVVVDVSHEDPEVKFNWYVDGVEVHNAKTKPREEQYNSTYRVVSVLTVLHQDWLNGKEYKCKVSNKALPAPIEKTISKAKGQPREPQVYTLPPSRDELTKNQVSLTCLVKGFYPSDIAVEWESNGQPENNYKTTPPVLDSDGSFFLYSKLTVDKSRWQQGNVFSCSVMHEGLHNPYTQKSLSLFPGK

SEQ ID NO: 63 - protein, 235 aa, Artificial Sequence
  Antibody 4 light chain
METPAQLLFLLLLWLPDTTGETVLTQSPGTLSLSPGERATLSCRASQSVSISYLAWYQRKPGQAPRLLIYGASRRATGIPDRFSGSGSGTDFTLTISRLEPEDFAVYYCQQYGSSPYTFGQGTKLEIKRTVAAPSVFIFPPSDEQLKSGTASVVCLLNNFYPREAKVQWKVDNALQSGNSQESVTEQDSKDSTYSLSSTLTLSKADYEKHKVYACEVTHQGLSSPVTKSFNRGEC

SEQ ID NO: 64 - protein, 476 aa, Artificial Sequence
  Antibody 4 heavy chain
MEFGLSWVFLVALLRGVQCQVQLVESGGGVVQPGRSLRLSCAASGFTFSRFGIHWVRQAPGKGLEWMAVIWYDGSNKFYADSVKGRFTISRDNSKNTVYLQMNSLRAEDTAVYYCAKDSRGYCSSIICFEGGLDNWGQGTLVTVSSASTKGPSVFPLAPSSKSTSGGTAALGCLVKDYFPEPVTVSWNSGALTSGVHTFPAVLQSSGLYSLSSVVTVPSSSLGTQTYICNVNHKPSNTKVDKRVEPKSCDKTHTCPPCPAPELLGGPSVFLFPPKPKDTLMISRTPEVTCVVVDVSHEDPEVKFNWYVDGVEVHNAKTKPREEQYNSTYRVVSVLTVLHQDWLNGKEYKCKVSNKALPAPIEKTISKAKGQPREPQVYTLPPSRDELTKNQVSLTCLVKGFYPSDIAVEWESNGQPENNYKTTPPVLDSDGSFFLYSKLTVDKSRWQQGNVFSCSVMHEGLHNHYTQKSLSLFPGK

SEQ ID NO: 65 - protein, 215 aa, Artificial Sequence
  Antibody 5 light chain
EIVLTQSPGTLSVSPGERATLSCRASRRVGSTYLAWYQQKPGQAPRRLIYGASSRAAGIPDRFSGTGSGTDFTLTISRVDPEDFAVYYCQQYAASPWTFGQGTTVEIKRTVAAPSVFIFPPSDEQLKSGTASVVCLLNNFYPREAKVQWKVDNALQSGNSQESVTEQDSKDSTYSLSSTLTLSKADYEKHKVYACEVTHQGLSSPVTKSFNRGEC

SEQ ID NO: 66 - protein, 456 aa, Artificial Sequence
  Antibody 5 heavy chain
QVQLVQSGGELKKPGASVRVSCKASGYTFTTYGISWVRQAPGQGLEWVGWISAYTGNTDYAQKVQGRVTMTTDTSTSTAYMELRSLTSDDTAVYYCARDKVQGRVEAGSGGRHDYWGQGTLVTVSSASTKGPSVFPLAPSSKSTSGGTAALGCLVKDYFPEPVTVSWNSGALTSGVHTFPAVLQSSGLYSLSSVVTVPSSSLGTQTYICNVNHKPSNTXVDKKVEPKSCDKTHTCPPCPAPELLGGPSVFLFPPKPKDTLMISRTPEVTCVVVDVSHEDPEVKFNWYVDGVEVHNAKTKPREEQYNSTYRVVSVLTVLHQDWLNGKEYKCKVSNKALPAPIEKTISKAKGQPREPQVYTLPPSRDELTKNQVSLTCLVKGFYPSDIAVEWESNGQPENNYKTTPPVLDSDGSFFLYSKLTVDKSRWQQGNVFSCSVMHEGLHNHYTQKSLSLSPGK

SEQ ID NO: 67 - protein, 215 aa, Artificial Sequence
  Antibody 6 light chain
EVVLTQSPGTLTLPPGDRATLSCRASHSVGSTYIAWFQQKSGQAPRRLIYGASNRATDIPDRFSGSGSGTDFTLTIRRLEPEDSAVYYCQQFSVSPWTFGQGTRVEIKRTVAAPSVFIFPPSDEQLKSGTASVVCLLNNFYPREAKVQWKVDNALQSGNSQESVTEQDSKDSTYSLSSTLTLSKADYEKHKVYACEVTHQGLSSPVTKSFNRGEC

SEQ ID NO: 68 - protein, 456 aa, Artificial Sequence
  Antibody 6 heavy chain
QVQLVQSGVEVKKPGASVKVSCKTSGYPFSTYGVSWVRQAPGQGLEWVGWISGYTGITDYAQKSQGRVTLTTDASTATAFLELRSLRPDDTATYFCARDKVQGRVEAGSGGRHDYWGQGTLVIVSSASTKGPSVFPLAPSSKSTSGGTAALGCLVKDYFPEPVTVSWNSGALTSGVHTFPAVLQSSGLYSLSSVVTVPSSSLGTQTYICNVNHKPSNTKVDKKVEPKSCDKTHTCPPCPAPELLGGPSVFLFPPKPKDTLMISRTPEVTCVVVDVSHEDPEVKFNWYVDGVEVHNAKTKPREEQYNSTYRVVSVLTVLHQDWLNGKEYKCKVSNKALPAPIEKTISKAKGQPREPQVYTLPPSRDELTKNQVSLTCLVKGFYPSDIAVEWESNGQPENNYKTTPPVLDSDGSFFLYSKLTVDKSRWQQGNVFSCSVMHEGLHNHYTQKSLSLSPGK

SEQ ID NO: 69 - protein, 215 aa, Artificial Sequence
  Antibody 7 light chain
EVVLTQSPGTLALPPGERATLSCRASHSIGSTYIAWYQQKSGQAPRRLIYGASNRASDIPDRFSGSGSGTDFTLTIRRLEPEDSAVYYCQQFSVSPWTFGQGTRVEIKRTVAAPSVFIFPPSDEQLKSGTASVVCLLNNFYPREAKVQWKVDNALQSGNSQESVTEQDSKDSTYSLSSTLTLSKADYEKHKVYACEVTHQGLSSPVTKSFNRGEC

SEQ ID NO: 70 - protein, 456 aa, Artificial Sequence
  Antibody 7 heavy chain
QVQLVQSGAEVKKPGASVKVSCKTSGYSFSTYGVSWVRQAPGQGLEWVGWISGYTGITDYAQKFQGRVTLTTDATTATAFLELRSLRPDDTATYFCARDKVQGRVEVGSGGRHDYWGQGTLVIVSSASTKGPSVFPLAPSSKSTSGGTAALGCLVKDYFPEPVTVSWNSGALTSGVHTFPAVLQSSGLYSLSSVVTVPSSSLGTQTYICNVNHKPSNTKVDKKVEPKSCDKTHTCPPCPAPELLGGPSVFLFPPKPKDTLMISRTPEVTCVVVDVSHEDPEVKFNWYVDGVEVHNAKTKPREEQYNSTYRVVSVLTVLHQDWLNGKEYKCKVSNKALPAPIEKTISKAKGQPREPQVYTLPPSRDELTKNQVSLTCLVKGFYPSDIAVEWESNGQPENNYKTTPPVLDSDGSFFLYSKLTVDKSRWQQGNVFSCSVMHEGLHNHYTQKSLSLSPGK

SEQ ID NO: 71 - DNA, 33 bp, Artificial Sequence
  Antibody 1 light chain CDR1
agggccagtgagaatatttggaacaacttggcc

SEQ ID NO: 72 - DNA, 21 bp, Artificial Sequence
  Antibody 1 light chain CDR2
ggtgcgtccaccggggccact

SEQ ID NO: 73 - DNA, 27 bp, Artificial Sequence
  Antibody 1 light chain CDR3
cagcagtataattcgtggcctcggacg

SEQ ID NO: 74 - DNA, 15 bp, Artificial Sequence
  Antibody 1 heavy chain CDR1
agtcatgctatcagt

SEQ ID NO: 75 - DNA, 51 bp, Artificial Sequence
  Antibody 1 heavy chain CDR2
gggatcagccctatgtttggaacaacacactacgcacagaagttccagggc

SEQ ID NO: 76 - DNA, 42 bp, Artificial Sequence
  Antibody 1 heavy chain CDR3
gatggtgcggggagttattatccactcaactggttcgacccc

SEQ ID NO: 77 - DNA, 36 bp, Artificial Sequence
  Antibody 2 light chain CDR1
agggccagtcaccgtgttggcagcacctacatagcc

SEQ ID NO: 78 - DNA, 21 bp, Artificial Sequence
  Antibody 2 light chain CDR2
ggtgcatccaacagggccact

SEQ ID NO: 79 - DNA, 27 bp, Artificial Sequence
  Antibody 2 light chain CDR3
cagcagtttagtgtttcaccgtggacg

SEQ ID NO: 80 - DNA, 15 bp, Artificial Sequence
  Antibody 2 heavy chain CDR1
acttatggagtcagt

SEQ ID NO: 81 - DNA, 51 bp, Artificial Sequence
  Antibody 2 heavy chain CDR2
tggatcagcgcttacactggtatcacagactacgcacagaagtttcagggc

SEQ ID NO: 82 - DNA, 51 bp, Artificial Sequence
  Antibody 2 heavy chain CDR3
gataaggtgcaggggcgcgttgaagtgggatctgggggtcgtcatgactac

SEQ ID NO: 83 - DNA, 36 bp, Artificial Sequence
  Antibody 3 light chain CDR1
agggccagtcagagtcttagcagcagctccttagtc

SEQ ID NO: 84 - DNA, 20 bp, Artificial Sequence
  Antibody 3 light chain CDR2
ggtgcatccagcagggccac

SEQ ID NO: 85 - DNA, 27 bp, Artificial Sequence
  Antibody 3 light chain CDR3
cagcagtatgggaactcaccgtacacg

SEQ ID NO: 86 - DNA, 18 bp, Artificial Sequence
  Antibody 3 heavy chain CDR1
aacaactatgctatcagc

SEQ ID NO: 87 - DNA, 54 bp, Artificial Sequence
  Antibody 3 heavy chain CDR2
ggagggatcagccctatctttgggacattaaactacgcagagaggttccagggc

SEQ ID NO: 88 - DNA, 33 bp, Artificial Sequence
  Antibody 3 heavy chain CDR3
ggttgtggctacaattgttactactttgacggg

SEQ ID NO: 89 - DNA, 36 bp, Artificial Sequence
  Antibody 4 light chain CDR1
agggccagtcagagtgttagcatcagctacttagcc

SEQ ID NO: 90 - DNA, 21 bp, Artificial Sequence
  Antibody 4 light chain CDR2
ggcgcatccaggagggccact

SEQ ID NO: 91 - DNA, 27 bp, Artificial Sequence
  Antibody 4 light chain CDR3
cagcagtatggtagctcaccgtacact

SEQ ID NO: 92 - DNA, 15 bp, Artificial Sequence
  Antibody 4 heavy chain CDR1
aggtttggcatccac

SEQ ID NO: 93 - DNA, 51 bp, Artificial Sequence
  Antibody 4 heavy chain CDR2
gttatatggtacgatggaagtaataaattctatgcagactccgtgaagggc

SEQ ID NO: 94 - DNA, 54 bp, Artificial Sequence
  Antibody 4 heavy chain CDR3
gattcccgcggatattgtagtagtatcatttgttttgaggggggacttgacaac

SEQ ID NO: 95 - DNA, 36 bp, Artificial Sequence
  Antibody 5 light chain CDR1
agggccagtcggcgcgttggcagcacctacttagcc

SEQ ID NO: 96 - DNA, 21 bp, Artificial Sequence
  Antibody 5 light chain CDR2
ggtgcatccagcagggccgct

SEQ ID NO: 97 - DNA, 27 bp, Artificial Sequence
  Antibody 5 light chain CDR3
cagcagtatgctgcctcaccgtggacg

SEQ ID NO: 98 - DNA, 15 bp, Artificial Sequence
  Antibody 5 heavy chain CDR1
acctatggcatcagc

SEQ ID NO: 99 - DNA, 51 bp, Artificial Sequence
  Antibody 5 heavy chain CDR2
tggatcagcgcttatactggaaatacagactatgcacagaaggtccagggc

SEQ ID NO: 100 - DNA, 51 bp, Artificial Sequence
  Antibody 5 heavy chain CDR3
gataaggtccaggggcgcgttgaagcgggaagtgggggccggcatgactac

SEQ ID NO: 101 - DNA, 36 bp, Artificial Sequence
  Antibody 6 light chain CDR1
agggccagtcacagtgttggcagcacctacatagcc

SEQ ID NO: 102 - DNA, 21 bp, Artificial Sequence
  Antibody 6 light chain CDR2
ggtgcatccaacagggccact

SEQ ID NO: 103 - DNA, 27 bp, Artificial Sequence
  Antibody 6 light chain CDR3
cagcagtttagtgtttcaccgtggacg

SEQ ID NO: 104 - DNA, 15 bp, Artificial Sequence
  Antibody 6 heavy chain CDR1
acttatggagtcagc

SEQ ID NO: 105 - DNA, 51 bp, Artificial Sequence
  Antibody 6 heavy chain CDR2
tggatcagcggttatactggtatcacagactacgcacagaagtctcagggc

SEQ ID NO: 106 - DNA, 51 bp, Artificial Sequence
  Antibody 6 heavy chain CDR3
gacaaagtgcaggggcgcgttgaagcgggatctgggggtcgtcacgactac

SEQ ID NO: 107 - DNA, 36 bp, Artificial Sequence
  Antibody 7 light chain CDR1
agggccagtcacagtattggcagcacctacatagcc

SEQ ID NO: 108 - DNA, 21 bp, Artificial Sequence
  Antibody 7 light chain CDR2
ggtgcatccaacagggcctct

SEQ ID NO: 109 - DNA, 27 bp, Artificial Sequence
  Antibody 7 light chain CDR3
cagcagtttagtgtttcaccgtggacg

SEQ ID NO: 110 - DNA, 15 bp, Artificial Sequence
  Antibody 7 heavy chain CDR1
acttatggagtcagc

SEQ ID NO: 111 - DNA, 51 bp, Artificial Sequence
  Antibody 7 heavy chain CDR2
tggatcagcggttacactggtatcacagactacgcacagaagtttcagggc

SEQ ID NO: 112 - DNA, 51 bp, Artificial Sequence; identical to SEQ ID NO: 82
  Antibody 7 heavy chain CDR3

SEQ ID NO: 113 - DNA, 381 bp, Artificial Sequence
  Antibody 1 light chain variable region
atggaagccccagctcagcttctcttcctcctgctactctggctcccagataccaccggagaaattgtgttgacacagtctccagccaccttgtctttgtctccaggggaaagagccaccctctcctgcagggccagtgagaatatttggaacaacttggcctggtaccagcaaaaacctggccaggctcccaggctcctcatctctggtgcgtccaccggggccactggtgtcccaagtaggtttagaggcagcgggtctaggacagaattcactctcaccatcagcagcctgcagtctgaagattttgcaatttatttctgtcagcagtataattcgtggcctcggacgttcggcccagggaccaaggtggagatcaaa

SEQ ID NO: 114 - DNA, 426 bp, Artificial Sequence
  Antibody 1 heavy chain variable region
atggactggacctggaggttcctctttgtggtggcagcagctacaggtgtccagtgccaggtgcagctggtgcagtctggggctgaggtgaagatgcctgggtcctcggtgaaggtctcctgcaagacttctggagtcttcttcagcagtcatgctatcagttgggtgcgacaggcccctggacaagggcttgagtggatgggagggatcagccctatgtttggaacaacacactacgcacagaagttccagggcagagtcacgattaccgcggaccaatccacgaccacagcctacatggagttgaccagtcttacatctgaggacacggccgtatattactgtgcgcgtgatggtgcggggagttattatccactcaactggttcgacccctggggccagggaaccctggtcaccgtctcctca

SEQ ID NO: 115 - DNA, 324 bp, Artificial Sequence
  Antibody 2 light chain variable region
gaagttgtgttgacacagtctcccggcaccctggctttgcctccaggggaaagagccaccctctcctgcagggccagtcaccgtgttggcagcacctacatagcctggtatcagcagaagtctggccaggctcccaggcgcctcatctatggtgcatccaacagggccactgacatcccagacaggttcagtggcagtgggtccgggacagacttcactctcaccatcaggagactggagcctgaagattctgcagtgtattactgtcagcagtttagtgtttcaccgtggacgttcggccaagggaccagggtggaaatcaag

SEQ ID NO: 116 - DNA, 378 bp, Artificial Sequence
  Antibody 2 heavy chain variable region
caggttcagctggtgcagtctggagctgaggtgaagaagcctggggcctcagtgaaggtctcctgcaagacttctggttattccttttccacttatggagtcagttgggtccgacaggcccccggacaagggcctgagtgggtgggatggatcagcgcttacactggtatcacagactacgcacagaagtttcagggcagagtcactctgaccacagacgcaaccacggccaccgccttcctggacctgaggagtctgagacctgacgacacggccacgtatttctgtgcgagagataaggtgcaggggcgcgttgaagtgggatctgggggtcgtcatgactactggggacagggaaccctggtcatcgtctcctca

SEQ ID NO: 117 - DNA, 384 bp, Artificial Sequence
  Antibody 3 light chain variable region
atggaaaccccagcgcagcttctcttcctcctgctactctggctcccagataccaccggagaaattgtgttgacgcagtctccaggcaccctgtctttgtctccaggggaaagagccaccctctcctgcagggccagtcagagtcttagcagcagctccttagtctggtaccagcagaaacctggccaggctcccaggctcctcatctatggtgcatccagcagggccactggcatcccagacaggttcagtggcagtgggtctgggacagacttcactctcaccatcagcagactggagcctgaagattttgcagtgtattactgtcagcagtatgggaactcaccgtacacgtttggccaggggacccaggttgagatcaaa

SEQ ID NO: 118 - DNA, 417 bp, Artificial Sequence
  Antibody 3 heavy chain variable region
atggactggacctggaggttcctctttgtggtggcagcagctacaggtgtccagtcccaggtgcagctggtgcagtctggggctgaggtgaagaagcctgggtcctcggtgaaggtctcctgcaaggcttctggaggcaccctcaacaactatgctatcagctgggtgcgacaggcccctggacaagggcttgagtggatgggagggatcagccctatctttgggacattaaactacgcagagaggttccagggcagagtcaccattaccgcggacgtatttacgaacacagtctacatggagctgagcagcctgagatctgaggacacggccgtgtatttctgtgcgagaggttgtggctacaattgttactactttgacgggtggggccagggaaccctggtcaccgtttcctca

SEQ ID NO: 119 - DNA, 384 bp, Artificial Sequence
  Antibody 4 light chain variable region
atggaaaccccagcgcagcttctcttcctcctgctactctggctcccagataccaccggagaaactgtgttgacgcagtctccaggcaccctgtctttgtctccaggggaaagagccaccctctcctgcagggccagtcagagtgttagcatcagctacttagcctggtaccagcggaaacctggccaggctcccaggctcctcatctatggcgcatccaggagggccactggcatcccagacaggttcagtggcagtgggtctgggacagacttcactctcaccatcagcagactggagcctgaagattttgcagtatattactgtcagcagtatggtagctcaccgtacacttttggccaggggaccaagctggagatcaaa

SEQ ID NO: 120 - DNA, 438 bp, Artificial Sequence
  Antibody 4 heavy chain variable region
atggagtttgggctgagctgggttttcctcgttgctcttttaagaggtgtccagtgtcaggtgcagctggtggagtctgggggaggcgtggtccagcctgggaggtccctgagactctcctgtgcagcgtctggattcaccttcagtaggtttggcatccactgggtccgccaggctccaggcaaggggctggagtggatggcagttatatggtacgatggaagtaataaattctatgcagactccgtgaagggccgattcaccatctccagagacaattccaagaacacggtttatctgcaaatgaacagcctcagagccgaggacacggctgtctattactgtgcgaaagattcccgcggatattgtagtagtatcatttgttttgaggggggacttgacaactggggccagggaaccctggtcaccgtctcctca

SEQ ID NO: 121 - DNA, 324 bp, Artificial Sequence
  Antibody 5 light chain variable region
gagattgtgttgactcagtctccaggcaccctgtctgtgtctccaggggaaagagccaccctctcctgcagggccagtcggcgcgttggcagcacctacttagcctggtaccagcagaaacctggccaggctcccaggcgcctcatctatggtgcatccagcagggccgctggcatcccagacaggttcagtggcactgggtctgggacagacttcactctcaccatcagcagggtggaccctgaagattttgcggtatattactgtcagcagtatgctgcctcaccgtggacgttcggccaagggaccacggtggagatcaaa

SEQ ID NO: 122 - DNA, 378 bp, Artificial Sequence
  Antibody 5 heavy chain variable region
caggttcagctggtgcagtctggaggtgagctgaagaagcctggggcctcagtgagggtctcctgtaaggcttctggctacacctttaccacctatggcatcagctgggtgcgacaggcccctggacaaggccttgagtgggtgggatggatcagcgcttatactggaaatacagactatgcacagaaggtccagggcagagtaaccatgaccacggacacatccacgagcacagcctacatggagctgaggagcctcacatctgacgacacggccgtctattactgtgcgagagataaggtccaggggcgcgttgaagcgggaagtgggggccggcatgactactggggccagggaaccctggtcaccgtctcctca

SEQ ID NO: 123 - DNA, 324 bp, Artificial Sequence
  Antibody 6 light chain variable region
gaagttgtgttgacgcagtctcccggcaccctgactttgcctccaggggacagagccaccctctcctgcagggccagtcacagtgttggcagcacctacatagcctggtttcagcagaagtctggccaggctcccaggcgcctcatctatggtgcatccaacagggccactgacatcccagacaggttcagtggcagtgggtccgggacagacttcactctcaccatcaggagactggagcctgaagattctgcagtgtactactgtcagcagtttagtgtttcaccgtggacgttcggccaagggaccagggtggaaatcaag

SEQ ID NO: 124 - DNA, 378 bp, Artificial Sequence
  Antibody 6 heavy chain variable region
caggttcagctggtccagtctggagtagaggtgaagaagcctggggcctcagtgaaggtctcctgcaagacttctggttatccgttttccacttatggagtcagctgggtccgacaggcccctggacaagggcttgagtgggtgggatggatcagcggttatactggtatcacagactacgcacagaagtctcagggcagagtcactctgacgacagacgcaagcacggccaccgccttcttggagctgaggagtctgaggcctgacgacacggccacctatttttgtgcgagagacaaagtgcaggggcgcgttgaagcgggatctgggggtcgtcacgactactggggacagggaaccctggtcatcgtctcctca

SEQ ID NO: 125 - DNA, 324 bp, Artificial Sequence
  Antibody 7 light chain variable region
gaagttgtgttgacgcagtctcccggcaccctggctttgcctccaggggaaagagccaccctctcctgcagggccagtcacagtattggcagcacctacatagcctggtatcagcagaagtctggccaggctcccaggcgcctcatctatggtgcatccaacagggcctctgacatcccagacaggttcagtggcagtgggtccgggacagacttcactctcaccatcaggagactggagcctgaagattctgcagtgtattactgtcagcagtttagtgtttcaccgtggacgttcggccaagggaccagggtggaaatcaag

SEQ ID NO: 126 - DNA, 378 bp, Artificial Sequence
  Antibody 7 heavy chain variable region
caggttcagctggtgcagtctggagctgaggtgaagaagcctggggcctcagtgaaggtctcctgcaagacttctggttattccttttccacttatggagtcagctgggtccgacaggcccctggacaagggcttgagtgggtgggatggatcagcggttacactggtatcacagactacgcacagaagtttcagggcagagtcactctgaccacagacgcaaccacggccaccgccttcctggagctgaggagtctgagacctgacgacacggccacctatttctgtgcgagagataaggtgcaggggcgcgttgaagtgggatctgggggtcgtcatgactactggggacagggaaccctggtcatcgtctcctca

SEQ ID NO: 127 - DNA, 705 bp, Artificial Sequence
  Antibody 1 light chain
atggaagccccagctcagcttctcttcctcctgctactctggctcccagataccaccggagaaattgtgttgacacagtctccagccaccttgtctttgtctccaggggaaagagccaccctctcctgcagggccagtgagaatatttggaacaacttggcctggtaccagcaaaaacctggccaggctcccaggctcctcatctctggtgcgtccaccggggccactggtgtcccaagtaggtttagaggcagcgggtctaggacagaattcactctcaccatcagcagcctgcagtctgaagattttgcaatttatttctgtcagcagtataattcgtggcctcggacgttcggcccagggaccaaggtggagatcaaacgaactgtggctgcaccatctgtcttcatcttcccgccatctgatgagcagttgaaatctggaactgcctctgttgtgtgcctgctgaataacttctatcccagagaggccaaagtacagtggaaggtggataacgccctccaatcgggtaactcccaggagagtgtcacagagcaggacagcaaggacagcacctacagcctcagcagcaccctgacgctgagcaaagcagactacgagaaacacaaagtctacgcctgcgaagtcacccatcagggcctgagctcgcccgtcacaaagagcttcaacaggggagagtgttag

SEQ ID NO: 128 - DNA, 1419 bp, Artificial Sequence
  Antibody 1 heavy chain
atggactggacctggaggttcctctttgtggtggcagcagctacaggtgtccagtgccaggtgcagctggtgcagtctggggctgaggtgaagatgcctgggtcctcggtgaaggtctcctgcaagacttctggagtcttcttcagcagtcatgctatcagttgggtgcgacaggcccctggacaagggcttgagtggatgggagggatcagccctatgtttggaacaacacactacgcacagaagttccagggcagagtcacgattaccgcggaccaatccacgaccacagcctacatggagttgaccagtcttacatctgaggacacggccgtatattactgtgcgcgtgatggtgcggggagttattatccactcaactggttcgacccctggggccagggaaccctggtcaccgtctcctcagcctccaccaagggcccatcggtcttccccctggcaccctcctccaagagcacctctgggggcacagcggccctgggctgcctggtcaaggactacttccccgaaccggtgacggtgtcgtggaactcaggcgccctgaccagcggcgtgcacaccttcccggctgtcctacagtcctcaggactctactccctcagcagcgtggtgaccgtgccctccagcagcttgggcacccagacctacatctgcaacgtgaatcacaagcccagcaacaccaaggtggacaagagagttgagcccaaatcttgtgacaaaactcacacatgcccaccgtgcccagcacctgaactcctggggggaccgtcagtcttcctcttccccccaaaacccaaggacaccctcatgatctcccggacccgtgaggtcacatgcgtggtggtggacgtgagccacgaagaccctgaggtcaagttcaactggtacgtggacggcgtggaggtgcataatgccaagacaaagccgcgggaggagcagtacaacagcacgtaccgtgtggtcagcgtcctcaccgtcctgcaccaggactggctgaatggcaaggagtacaagtgcaaggtctccaacaaagccctcccagcccccatcgagaaaaccatctccaaagccaaagggcagccccgagaaccacaggtgtacaccctgcccccatcccgggatgagctgaccaagaaccaggtcagcctgacctgcctggtcaaaggcttttatcccagcgacatcgccgtggagtgggagagcaatgggcagccggagaacaactacaagaccacgcctcccgtgctggactccgacggctcctttttcctttacagcaagctcaccgtggacaagagcaggtggcagcaggggaacgttttttcatgctccgtgatgcatgagggtttgcacaaccactacacgcagaagagcctctccctgtttccgggtaaatga

SEQ ID NO: 129 - DNA, 648 bp, Artificial Sequence
  Antibody 2 light chain
gaagttgtgttgacacagtctcccggcaccctggctttgcctccaggggaaagagccaccctctcctgcagggccagtcaccgtgttggcagcacctacatagcctggtatcagcagaagtctggccaggctcccaggcgcctcatctatggtgcatccaacagggccactgacatcccagacaggttcagtggcagtgggtccgggacagacttcactctcaccatcaggagactggagcctgaagattctgcagtgtattactgtcagcagtttagtgtttcaccgtggacgttcggccaagggaccagggtggaaatcaagcgaactgtggctgcaccatctgtcttcatcttcccgccatctgatgagcagttgaaatctggaactgcctctgttgtgtgcctgctgaataacttctatcccagagaggccaaagtacagtggaaggtggataacgccctccaatcgggtaactcccaggagagtgtcacagagcaggacagcaaggacagcacctacagcctcagcagcaccctgacgctgagcaaagcagactacgagaaacacaaagtctacgcctgcgaagtcacccatcagggcctgagctcgcccgtcacaaagagcttcaacaggggagagtgttag

SEQ ID NO: 130 - DNA, 1371 bp, Artificial Sequence
  Antibody 2 heavy chain
caggttcagctggtgcagtctggagctgaggtgaagaagcctggggcctcagtgaaggtctcctgcaagacttctggttattccttttccacttatggagtcagttgggtccgacaggcccccggacaagggcctgagtgggtgggatggatcagcgcttacactggtatcacagactacgcacagaagtttcagggcagagtcactctgaccacagacgcaaccacggccaccgccttcctggacctgaggagtctgagacctgacgacacggccacgtatttctgtgcgagagataaggtgcaggggcgcgttgaagtgggatctgggggtcgtcatgactactggggacagggaaccctggtcatcgtctcctcagcctccaccaagggcccatcggtcttccccctggcaccctcctccaagagcacctctgggggcacagcggccctgggctgcctggtcaaggactacttccccgaaccggtgacggtgtcgtggaactcaggcgccctgaccagcggcgtgcacaccttcccggctgtcctacagtcctcaggactctactccctcagcagcgtggtgaccgtgccctccagcagcttgggcacccagacctacatctgcaacgtgaatcacaagcccagcaacaccaaggtggacaagaaagttgagcccaaatcttgtgacaaaactcacacatgcccaccgtgcccagcacctgaactcctggggggaccgtcagtcttcctcttccccccaaaacccaaggacaccctcatgatctcccggacccctgaggtcacatgcgtggtggtggacgtgagccacgaagaccctgaggtcaagttcaactggtacgtggacggcgtggaggtgcataatgccaagacaaagccgcgggaggagcagtacaacagcacgtaccgtgtggtcagcgtcctcaccgtcctgcaccaggactggctgaatggcaaggagtacaagtgcaaggtctccaacaaagccctcccagcccccatcgagaaaaccatctccaaagccaaagggcagccccgagaaccacaggtgtacaccctgcccccatcccgggatgagctgaccaagaaccaggtcagcctgacctgcctggtcaaaggcttctatcccagcgacatcgccgtggagtgggagagcaatgggcagccggagaacaactacaagaccacgcctcccgtgctggactccgacggctccttcttcctctacagcaagctcaccgtggacaagagcaggtggcagcaggggaacgtcttctcatgctccgtgatgcatgagggtctgcacaaccactacacgcagaagagcctctccctgtctccgggtaaatga

SEQ ID NO: 131 - DNA, 708 bp, Artificial Sequence
  Antibody 3 light chain
atggaaaccccagcgcagcttctcttcctcctgctactctggctcccagataccaccggagaaattgtgttgacgcagtctccaggcaccctgtctttgtctccaggggaaagagccaccctctcctgcagggccagtcagagtcttagcagcagctccttagtctggtaccagcagaaacctggccaggctcccaggctcctcatctatggtgcatccagcagggccactggcatcccagacaggttcagtggcagtgggtctgggacagacttcactctcaccatcagcagactggagcctgaagattttgcagtgtattactgtcagcagtatgggaactcaccgtacacgtttggccaggggacccaggttgagatcaaacgaactgtggctgcaccatctgtcttcatcttcccgccatctgatgagcagttgaaatctggaactgcctctgttgtgtgcctgctgaataacttctatcccagagaggccaaagtacagtggaaggtggataacgccctccaatcgggtaactcccaggagagtgtcacagagcaggacagcaaggacagcacctacagcctcagcagcaccctgacgctgagcaaagcagactacgagaaacacaaagtctacgcctgcgaagtcacccatcagggcctgagctcgcccgtcacaaagagcttcaacaggggagagtgttag

SEQ ID NO: 132 - DNA, 1410 bp, Artificial Sequence
  Antibody 3 heavy chain
atggactggacctggaggttcctctttgtggtggcagcagctacaggtgtccagtcccaggtgcagctggtgcagtctggggctgaggtgaagaagcctgggtcctcggtgaaggtctcctgcaaggcttctggaggcaccctcaacaactatgctatcagctgggtgcgacaggcccctggacaagggcttgagtggatgggagggatcagccctatctttgggacattaaactacgcagagaggttccagggcagagtcaccattaccgcggacgtatttacgaacacagtctacatggagctgagcagcctgagatctgaggacacggccgtgtatttctgtgcgagaggttgtggctacaattgttactactttgacgggtggggccagggaaccctggtcaccgtttcctcagcctccaccaagggcccatcggtcttccccctggcaccctcctccaagagcacctctgggggcacagcggccctgggctgcctggtcaaggactacttccccgaaccggtgacggtgtcgtggaactcaggcgccctgaccagcggcgtgcacaccttcccggctgtcctacagtcctcaggactctactccctcagcagcgtggtgaccgtgccctccagcagcttgggcacccagacctacatctgcaacgtgaatcacaagcccagcaacaccaaggtggacaagaaagttgagcccaaatcttgtgacaaaactcacacatgcccaccgtgcccagcacctgaactcctggggggaccgtcagtcttcctcttccccccaaaacccaaggacaccctcatgatctcccggacccctgaggtcacatgcgtggtggtggacgtgagccacgaagaccctgaggtcaagttcaactggtacgtggacggcgtggaggtgcataatgccaagacaaagccgcgggaggagcagtacaacagcacgtaccgtgtggtcagcgtcctcaccgtcctgcaccaggactggctgaatggcaaggagtacaagtgcaaggtctccaacaaagccctcccagcccccatcgagaaaaccatctccaaagccaaagggcagccccgagaaccacaggtgtacaccctgcccccatcccgggatgagctgaccaagaaccaggtcagcctgacctgcctggtcaaaggcttctatcccagcgacatcgccgtggagtgggagagcaatgggcagccggagaacaactacaagaccacgcctcccgtgctggactccgacggctcctttttcctttacagcaagctcaccgtggacaagagcaggtggcagcaggggaacgttttttcatgctccgtgatgcatgagggtttgcacaacccctacacgcagaagagcctctccctgtttccgggtaaatga

SEQ ID NO: 133 - DNA, 708 bp, Artificial Sequence
  Antibody 4 light chain
atggaaaccccagcgcagcttctcttcctcctgctactctggctcccagataccaccggagaaactgtgttgacgcagtctccaggcaccctgtctttgtctccaggggaaagagccaccctctcctgcagggccagtcagagtgttagcatcagctacttagcctggtaccagcggaaacctggccaggctcccaggctcctcatctatggcgcatccaggagggccactggcatcccagacaggttcagtggcagtgggtctgggacagacttcactctcaccatcagcagactggagcctgaagattttgcagtatattactgtcagcagtatggtagctcaccgtacacttttggccaggggaccaagctggagatcaaacgaactgtggctgcaccatctgtcttcatcttcccgccatctgatgagcagttgaaatctggaactgcctctgttgtgtgcctgctgaataacttctatcccagagaggccaaagtacagtggaaggtggataacgccctccaatcgggtaactcccaggagagtgtcacagagcaggacagcaaggacagcacctacagcctcagcagcaccctgacgctgagcaaagcagactacgagaaacacaaagtctacgcctgcgaagtcacccatcagggcctgagctcgcccgtcacaaagagcttcaacaggggagagtgttag

SEQ ID NO: 134 - DNA, 1431 bp, Artificial Sequence
  Antibody 4 heavy chain
atggagtttgggctgagctgggttttcctcgttgctcttttaagaggtgtccagtgtcaggtgcagctggtggagtctgggggaggcgtggtccagcctgggaggtccctgagactctcctgtgcagcgtctggattcaccttcagtaggtttggcatccactgggtccgccaggctccaggcaaggggctggagtggatggcagttatatggtacgatggaagtaataaattctatgcagactccgtgaagggccgattcaccatctccagagacaattccaagaacacggtttatctgcaaatgaacagcctcagagccgaggacacggctgtctattactgtgcgaaagattcccgcggatattgtagtagtatcatttgttttgaggggggacttgacaactggggccagggaaccctggtcaccgtctcctcagcctccaccaagggcccatcggtcttccccctggcaccctcctccaagagcacctctgggggcacagcggccctgggctgcctggtcaaggactacttccccgaaccggtgacggtgtcgtggaactcaggcgccctgaccagcggcgtgcacaccttcccggctgtcctacagtcctcaggactctactccctcagcagcgtggtgaccgtgccctccagcagcttgggcacccagacctacatctgcaacgtgaatcacaagcccagcaacaccaaggtggacaagagagttgagcccaaatcttgtgacaaaactcacacatgcccaccgtgcccagcacctgaactcctggggggaccgtcagtcttcctcttccccccaaaacccaaggacaccctcatgatctcccggacccctgaggtcacatgcgtggtggtggacgtgagccacgaagaccctgaggtcaagttcaactggtacgtggacggcgtggaggtgcataatgccaagacaaagccgcgggaggagcagtacaacagcacgtaccgtgtggtcagcgtcctcaccgtcctgcaccaggactggctgaatggcaaggagtacaagtgcaaggtctccaacaaagccctcccagcccccatcgagaaaaccatctccaaagccaaagggcagccccgagaaccacaggtgtacaccctgcccccatcccgggatgagctgaccaagaaccaggtcagcctgacctgcctggtcaaaggcttctatcccagcgacatcgccgtggagtgggagagcaatgggcagccggagaacaactacaagaccacgcctcccgtgctggactccgacggctcctttttcctttacagcaagctcaccgtggacaagagcaggtggcagcaggggaacgtcttttcatgctccgtgatgcatgagggtttgcacaaccactacacgcagaagagcctctccctgtttccgggtaaatga

SEQ ID NO: 135 - DNA, 648 bp, Artificial Sequence
  Antibody 5 light chain
gagattgtgttgactcagtctccaggcaccctgtctgtgtctccaggggaaagagccaccctctcctgcagggccagtcggcgcgttggcagcacctacttagcctggtaccagcagaaacctggccaggctcccaggcgcctcatctatggtgcatccagcagggccgctggcatcccagacaggttcagtggcactgggtctgggacagacttcactctcaccatcagcagggtggaccctgaagattttgcggtatattactgtcagcagtatgctgcctcaccgtggacgttcggccaagggaccacggtggagatcaaacgaactgtggctgcaccatctgtcttcatcttcccgccatctgatgagcagttgaaatctggaactgcctctgttgtgtgcctgctgaataacttctatcccagagaggccaaagtacagtggaaggtggataacgccctccaatcgggtaactcccaggagagtgtcacagagcaggacagcaaggacagcacctacagcctcagcagcaccctgacgctgagcaaagcagactacgagaaacacaaagtctacgcctgcgaagtcacccatcagggcctgagctcgcccgtcacaaagagcttcaacaggggagagtgttag

SEQ ID NO: 136 - DNA, 1371 bp, Artificial Sequence
  Antibody 5 heavy chain
caggttcagctggtgcagtctggaggtgagctgaagaagcctggggcctcagtgagggtctcctgtaaggcttctggctacacctttaccacctatggcatcagctgggtgcgacaggcccctggacaaggccttgagtgggtgggatggatcagcgcttatactggaaatacagactatgcacagaaggtccagggcagagtaaccatgaccacggacacatccacgagcacagcctacatggagctgaggagcctcacatctgacgacacggccgtctattactgtgcgagagataaggtccaggggcgcgttgaagcgggaagtgggggccggcatgactactggggccagggaaccctggtcaccgtctcctcagcctccaccaagggcccatcggtcttccccctggcaccctcctccaagagcacctctgggggcacagcggccctgggctgcctggtcaaggactacttccccgaaccggtgacggtgtcgtggaactcaggcgccctgaccagcggcgtgcacaccttcccggctgtcctacagtcctcaggactctactctctcagcagcgtggtgaccgtgccctccagcagcttgggcacccagacctacatctgcaacgtgaatcacaagcccagcaacaccaargtggacaagaaagttgagcccaaatcttgtgacaaaactcacacatgcccaccgtgcccagcacctgaactcctggggggaccgtcagtcttcctcttccccccaaaacccaaggacaccctcatgatctcccggacccctgaggtcacatgcgtggtggtggacgtgagccacgaagaccctgaggtcaagttcaactggtacgtggacggcgtggaggtgcataatgccaagacaaagccgcgggaggagcagtacaacagcacgtaccgtgtggtcagcgtcctcaccgtcctgcaccaggactggctgaatggcaaggagtacaagtgcaaggtctccaacaaagccctcccagcccccatcgagaaaaccatctccaaagccaaagggcagccccgagaaccacaggtgtacaccctgcccccatcccgggatgagctgaccaagaaccaggtcagcctgacctgcctggtcaaaggcttctatcccagcgacatcgccgtggagtgggagagcaatgggcagccggagaacaactacaagaccacgcctcccgtgctggactccgacggctccttcttcctctacagcaagctcaccgtggacaagagcaggtggcagcaggggaacgtcttctcatgctccgtgatgcatgagggtctgcacaaccactacacgcagaagagcctctccctgtctccgggtaaatga

SEQ ID NO: 137 - DNA, 648 bp, Artificial Sequence
  Antibody 6 light chain
gaagttgtgttgacgcagtctcccggcaccctgactttgcctccaggggacagagccaccctctcctgcagggccagtcacagtgttggcagcacctacatagcctggtttcagcagaagtctggccaggctcccaggcgcctcatctatggtgcatccaacagggccactgacatcccagacaggttcagtggcagtgggtccgggacagacttcactctcaccatcaggagactggagcctgaagattctgcagtgtactactgtcagcagtttagtgtttcaccgtggacgttcggccaagggaccagggtggaaatcaagcgaactgtggctgcaccatctgtcttcatcttcccgccatctgatgagcagttgaaatctggaactgcctctgttgtgtgcctgctgaataacttctatcccagagaggccaaagtacagtggaaggtggataacgccctccaatcgggtaactcccaggagagtgtcacagagcaggacagcaaggacagcacctacagcctcagcagcaccctgacgctgagcaaagcagactacgagaaacacaaagtctacgcctgcgaagtcacccatcagggcctgagctcgcccgtcacaaagagcttcaacaggggagagtgttag

SEQ ID NO: 138 - DNA, 1371 bp, Artificial Sequence
  Antibody 6 heavy chain
caggttcagctggtccagtctggagtagaggtgaagaagcctggggcctcagtgaaggtctcctgcaagacttctggttatccgttttccacttatggagtcagctgggtccgacaggcccctggacaagggcttgagtgggtgggatggatcagcggttatactggtatcacagactacgcacagaagtctcagggcagagtcactctgacgacagacgcaagcacggccaccgccttcttggagctgaggagtctgaggcctgacgacacggccacctatttttgtgcgagagacaaagtgcaggggcgcgttgaagcgggatctgggggtcgtcacgactactggggacagggaaccctggtcatcgtctcctcagcctccaccaagggcccatcggtcttccccctggcaccctcctccaagagcacctctgggggcacagcggccctgggctgcctggtcaaggactacttccccgaaccggtgacggtgtcgtggaactcaggcgccctgaccagcggcgtgcacaccttcccggctgtcctacagtcctcaggactctactccctcagcagcgtggtgaccgtgccctccagcagcttgggcacccagacctacatctgcaacgtgaatcacaagcccagcaacaccaaggtggacaagaaagttgagcccaaatcttgtgacaaaactcacacatgcccaccgtgcccagcacctgaactcctggggggaccgtcagtcttcctcttccccccaaaacccaaggacaccctcatgatctcccggacccctgaggtcacatgcgtggtggtggacgtgagccacgaagaccctgaggtcaagttcaactggtacgtggacggcgtggaggtgcataatgccaagacaaagccgcgggaggagcagtacaacagcacgtaccgtgtggtcagcgtcctcaccgtcctgcaccaggactggctgaatggcaaggagtacaagtgcaaggtctccaacaaagccctcccagcccccatcgagaaaaccatctccaaagccaaagggcagccccgagaaccacaggtgtacaccctgcccccatcccgggatgagctgaccaagaaccaggtcagcctgacctgcctggtcaaaggcttctatcccagcgacatcgccgtggagtgggagagcaatgggcagccggagaacaactacaagaccacgcctcccgtgctggactccgacggctccttcttcctctacagcaagctcaccgtggacaagagcaggtggcagcaggggaacgtcttctcatgctccgtgatgcatgagggtctgcacaaccactacacgcagaagagcctctccctgtctccgggtaaatga

SEQ ID NO: 139 - DNA, 648 bp, Artificial Sequence
  Antibody 7 light chain
gaagttgtgttgacgcagtctcccggcaccctggctttgcctccaggggaaagagccaccctctcctgcagggccagtcacagtattggcagcacctacatagcctggtatcagcagaagtctggccaggctcccaggcgcctcatctatggtgcatccaacagggcctctgacatcccagacaggttcagtggcagtgggtccgggacagacttcactctcaccatcaggagactggagcctgaagattctgcagtgtattactgtcagcagtttagtgtttcaccgtggacgttcggccaagggaccagggtggaaatcaagcgaactgtggctgcaccatctgtcttcatcttcccgccatctgatgagcagttgaaatctggaactgcctctgttgtgtgcctgctgaataacttctatcccagagaggccaaagtacagtggaaggtggataacgccctccaatcgggtaactcccaggagagtgtcacagagcaggacagcaaggacagcacctacagcctcagcagcaccctgacgctgagcaaagcagactacgagaaacacaaagtctacgcctgcgaagtcacccatcagggcctgagctcgcccgtcacaaagagcttcaacaggggagagtgttag

SEQ ID NO: 140 - DNA, 1371 bp, Artificial Sequence
  Antibody 7 heavy chain
caggttcagctggtgcagtctggagctgaggtgaagaagcctggggcctcagtgaaggtctcctgcaagacttctggttattccttttccacttatggagtcagctgggtccgacaggcccctggacaagggcttgagtgggtgggatggatcagcggttacactggtatcacagactacgcacagaagtttcagggcagagtcactctgaccacagacgcaaccacggccaccgccttcctggagctgaggagtctgagacctgacgacacggccacctatttctgtgcgagagataaggtgcaggggcgcgttgaagtgggatctgggggtcgtcatgactactggggacagggaaccctggtcatcgtctcctcagcctccaccaagggcccatcggtcttccccctggcaccctcctccaagagcacctctgggggcacagcggccctgggctgcctggtcaaggactacttccccgaaccggtgacggtgtcgtggaactcaggggccctgaccagcggcgtgcacaccttcccggctgtcctacagtcctcaggactctactccctcagcagcgtggtgaccgtgccctccagcagcttgggcacccagacctacatctgcaacgtgaatcacaagcccagcaacaccaaggtggacaagaaagttgagcccaaatcttgtgacaaaactcacacatgcccaccgtgcccagcacctgaactcctggggggaccgtcagtcttcctcttccccccaaaacccaaggacaccctcatgatctcccggacccctgaggtcacatgcgtggtggtggacgtgagccacgaagaccctgaggtcaagttcaactggtacgtggacggcgtggaggtgcataatgccaagacaaagccgcgggaggagcagtacaacagcacgtaccgtgtggtcagcgtcctcaccgtcctgcaccaggactggctgaatggcaaggagtacaagtgcaaggtctccaacaaagccctcccagcccccatcgagaaaaccatctccaaagccaaagggcagccccgagaaccacaggtgtacaccctgcccccatcccgggatgagctgaccaagaaccaggtcagcctgacctgcctggtcaaaggcttctatcccagcgacatcgccgtggagtgggagagcaatgggcagccggagaacaactacaagaccacgcctcccgtgctggactccgacggctccttcttcctctacagcaagctcaccgtggacaagagcaggtggcagcaggggaacgtcttctcatgctccgtgatgcatgagggtctgcacaaccactacacgcagaagagcctctccctgtctccgggtaaatga